European Patent Application EP 4 545 556 A1, published April 30, 2025. Title: Production of recombinant proteins. Applicant: Real Deal Milk S.L. Application EP. The sequence listing filed with the application follows.

SEQUENCE LISTING (24 sequences)

SEQ ID NO: 1 - protein, 162 aa, Bos taurus
LIVTQTMKGLDIQKVAGTWYSLAMAASDISLLDAQSAPLRVYVEELKPTPEGDLEILLQKWENGECAQKKIIAEKTKIPAVFKIDALNENKVLVLDTDYKKYLLFCMENSAEPEQSLACQCLVRTPEVDDEALEKFDKALKALPMHIRLSFNPTQLEEQCHI

SEQ ID NO: 2 - protein, 14 aa, Bos taurus
HPHPHLSFMAIPPK

SEQ ID NO: 3 - protein, 27 aa, synthetic construct
  SITE 1: note = X is A or I or L or V
  SITE 4: note = X is D or E
  SITE 6..8: note = X is S or T
  SITE 11: note = X is A or I or L or V
  SITE 12: note = X is D or E
  SITE 13..14: note = X is A or I or L or V
  SITE 15: note = X is D or E
  SITE 17: note = X is S or T
  SITE 18..19: note = X is A or I or L or V
  SITE 20: note = X is S or T
  SITE 21: note = X is A or I or L or V
  SITE 22: note = X is D or E
  SITE 23: note = X iS A or I or L or V
  SITE 24: note = X is S or T
  SITE 26: note = X is D or E
  SITE 27: note = X is A or I or L or V
XSGXPXXXPTXXXXXSXXXXXXXXPXX

SEQ ID NO: 4 - protein, 44 aa, synthetic construct
  SITE 1: note = X is A, L, I or V
  SITE 4: note = X is D or E
  SITE 6..8: note = X is S or T
  SITE 11: note = X is A, I, L or V
  SITE 12: note = X is D or E
  SITE 13..14: note = X is A, I, L or V
  SITE 15: note = X is D or E
  SITE 17: note = X is S or T
  SITE 18..19: note = X is A, I, L or V
  SITE 20: note = X is S or T
  SITE 22: note = X is D or E
  SITE 24: note = X is S or T
  SITE 27..28: note = X is A, I, L, or V
  SITE 21: note = Xis A, I, L or V
  SITE 23: note = X is A, I, L or V
  SITE 26: note = X is D or E
  SITE 29: note = X is D or E
  SITE 33: note = X is D or E
  SITE 34: note = X is A, I, L or V
  SITE 37: note = X is A, I, L or V
  SITE 39: note = X is A, I, L or V
  SITE 40: note = X is S or T
  SITE 43..44: note = X is A, I, L or V
XSGXPXXXPTXXXXXSXXXXXXXXPXXXXSPPXXNTXQXXSTXX

SEQ ID NO: 5 - protein, 41 aa, synthetic construct
  SITE 4: note = X is D or E
  SITE 7: note = X is D or E
  SITE 8: note = X is A, I, L or V
  SITE 10: note = X is S or T
  SITE 11: note = X is A, I, L or V
  SITE 14..15: note = X is A, I, L or V
  SITE 18: note = X is D or E
  SITE 20..22: note = X is S or T
  SITE 25: note = X is A, I, L or V
  SITE 26: note = X is D or E
  SITE 27..28: note = X is A, I, L or V
  SITE 29: note = X is D or E
  SITE 31: note = X is S or T
  SITE 32..33: note = X is A, I, L or V
  SITE 34: note = X is S or T
  SITE 35: note = X is A, I, L or V
  SITE 36: note = X is D or E
  SITE 37: note = X is A, I, L or V
  SITE 38: note = X is S or T
  SITE 40: note = X is D or E
  SITE 41: note = X is A, I, L or V
KNQXKTXXPXXNTXXSGXPXXXPTXXXXXSXXXXXXXXPXX

SEQ ID NO: 6 - protein, 58 aa, synthetic construct
  SITE 4: note = X is D or E
  SITE 7: note = X is D or E
  SITE 8: note = X is A, I, L or V
  SITE 10: note = X is S or T
  SITE 11: note = X is A, I, L, or V
  SITE 14..15: note = X is A, I, L, or V
  SITE 18: note = X is D or E
  SITE 20..22: note = X is S or T
  SITE 25: note = X is A, I, L or V
  SITE 26: note = X is D or E
  SITE 27..28: note = X is A, I, L or V
  SITE 29: note = X is D or E
  SITE 31: note = X is S or T
  SITE 32..33: note = X is A, I, L or V
  SITE 34: note = X is S or T
  SITE 35: note = X is A, I, L or V
  SITE 36: note = X is D or E
  SITE 37: note = X is A, I, L or V
  SITE 38: note = X is S or T
  SITE 40: note = X is D or E
  SITE 41: note = X is A, I, L or V
  SITE 42: note = X is A, I, L or V
  SITE 43: note = X is D or E
  SITE 47: note = X is D or E
  SITE 48: note = X is A, I, L, or V
  SITE 51: note = X is A, I, L or V
  SITE 53: note = X is A, I, L or V
  SITE 54: note = X is S or T
  SITE 57..58: note = X is A, I, L or V
KNQXKTXXPXXNTXXSGXPXXXPTXXXXXSXXXXXXXXPXXXXSPPXXNTXQXXSTXX

SEQ ID NO: 7 - protein, 27 aa, synthetic construct
ASGEPTSTPTIEAVESTVATLEASPEV

SEQ ID NO: 8 - protein, 44 aa, synthetic construct
ASGEPTSTPTIEAVESTVATLEASPEVIESPPEINTVQVTSTAV

SEQ ID NO: 9 - protein, 41 aa, synthetic construct
KNQDKTEIPTINTIASGEPTSTPTIEAVESTVATLEASPEV

SEQ ID NO: 10 - protein, 58 aa, synthetic construct
KNQDKTEIPTINTIASGEPTSTPTIEAVESTVATLEASPEVIESPPEINTVQVTSTAV

SEQ ID NO: 11 - protein, 8 aa, synthetic construct
  SITE 5: note = X is L, M or F
HLSFXAIP

SEQ ID NO: 12 - protein, 14 aa, synthetic construct
  SITE 14: note = X is W, Y, F, C, R, I, M, H, L, V, K, N, T or A
FLQKQQYGISSKFX

SEQ ID NO: 13 - protein, 14 aa, synthetic construct
RPRPRPSFIAIPPK

SEQ ID NO: 14 - protein, 89 aa, synthetic construct
MRFPSIFTAVLFAASSALAAPVNTTTEDETAQIPAEAVIGYSDLEGDFDVAVLPFSNSTNNGLLFINTTIASIAAKEEGVSLEKREAEA

SEQ ID NO: 15 - protein, 319 aa, synthetic construct
MRFPSIFTAVLFAASSALAAPVNTTTEDETAQIPAEAVIGYSDLEGDFDVAVLPFSASIAAKEEGVSLEKREAEALIVTQTMKGLDIQKVAGTWYSLAMAASDISLLDAQSAPLRVYVEELKPTPEGDLEILLQKWENGECAQKKIIAEKTKIPAVFKIDALNENKVLVLDTDYKKYLLFCMENSAEPEQSLACQCLVRTPEVDDEALEKFDKALKALPMHIRLSFNPTQLEEQCHIHPHPHLSFMAIPPKKNQDKTEIPTINTIASGEPTSTPTIEAVESTVATLEASPEVIESPPEINTVQVTSTAVGSGSHHHHHH

SEQ ID NO: 16 - protein, 248 aa, synthetic construct
EAEALIVTQTMKGLDIQKVAGTWYSLAMAASDISLLDAQSAPLRVYVEELKPTPEGDLEILLQKWENGECAQKKIIAEKTKIPAVFKIDALNENKVLVLDTDYKKYLLFCMENSAEPEQSLACQCLVRTPEVDDEALEKFDKALKALPMHIRLSFNPTQLEEQCHIHPHPHLSFMAIPPKKNQDKTEIPTINTIASGEPTSTPTIEAVESTVATLEASPEVIESPPEINTVQVTSTAVGSGSHHHHHH

SEQ ID NO: 17 - protein, 239 aa, synthetic construct
EAEALIVTQTMKGLDIQKVAGTWYSLAMAASDISLLDAQSAPLRVYVEELKPTPEGDLEILLQKWENGECAQKKIIAEKTKIPAVFKIDALNENKVLVLDTDYKKYLLFCMENSAEPEQSLACQCLVRTPEVDDEALEKFDKALKALPMHIRLSFNPTQLEEQCHIDDDDKKNQDKTEIPTINTIASGEPTSTPTIEAVESTVATLEASPEVIESPPEINTVQVTSTAVGSGSHHHHHH

SEQ ID NO: 18 - DNA, 960 bp, synthetic construct
  source 1..960: mol_type = other DNA
atgagatttccatctattttcactgctgttttgtttgctgcttcttctgctttggctgctccagttaacactactactgaagatgagactgctcaaattcctgctgaagctgttattggttactctgatttggagggagattttgatgttgctgttttgcctttctctgcttctatcgctgctaaggaagagggtgtttctttggaaaagagagaagctgaggctttgattgttactcaaactatgaagggtttggatatccaaaaggttgctggtacttggtactctttggctatggctgcttctgatatttctttgttggatgctcaatctgctccattgagagtttatgttgaagagttgaaaccaactcctgaaggagatttggaaattttgttgcaaaagtgggaaaacggagagtgtgctcaaaagaaaattatcgctgaaaagactaagatccctgctgtttttaaaatcgatgctttgaacgagaataaggttttggttttggatactgattacaagaaatatttgttgttctgtatggaaaactctgctgaaccagagcaatctttggcttgtcaatgtttggttagaactcctgaagttgatgatgaagctttggagaagtttgataaagctttgaaggctttgccaatgcatatcagattgtctttcaatcctactcaattggaagagcaatgtcacattcatccacaccctcatttgtctttcatggctattccacctaagaaaaaccaagataagactgaaatcccaactattaatactattgcttctggagagccaacttctactcctactattgaagctgttgagtctactgttgctactttggaagcttctcctgaagttattgagtctccacctgagattaatactgttcaagttacttctactgctgttggttctggatcccatcaccatcaccatcactaa

SEQ ID NO: 19 - DNA, 933 bp, synthetic construct
  source 1..933: mol_type = other DNA
atgagatttccatctattttcactgctgttttgtttgctgcttcttctgctttggctgctccagttaacactactactgaagatgagactgctcaaattcctgctgaagctgttattggttactctgatttggagggagattttgatgttgctgttttgcctttctctgcttctatcgctgctaaggaagagggtgtttctttggaaaagagagaagctgaggctttgattgttactcaaactatgaagggtttggatatccaaaaggttgctggtacttggtactctttggctatggctgcttctgatatttctttgttggatgctcaatctgctccattgagagtttatgttgaagagttgaaaccaactcctgaaggagatttggaaattttgttgcaaaagtgggaaaacggagagtgtgctcaaaagaaaattatcgctgaaaagactaagatccctgctgtttttaaaatcgatgctttgaacgagaataaggttttggttttggatactgattacaagaaatatttgttgttctgtatggaaaactctgctgaaccagagcaatctttggcttgtcaatgtttggttagaactcctgaagttgatgatgaagctttggagaagtttgataaagctttgaaggctttgccaatgcatatcagattgtctttcaatcctactcaattggaagagcaatgtcacattgatgacgatgacaagaaaaaccaagataagactgaaatcccaactattaatactattgcttctggagagccaacttctactcctactattgaagctgttgagtctactgttgctactttggaagcttctcctgaagttattgagtctccacctgagattaatactgttcaagttacttctactgctgttggttctggatcccatcaccatcaccatcactaa

SEQ ID NO: 20 - protein, 174 aa, synthetic construct
EAEALIVTQTMKGLDIQKVAGTWYSLAMAASDISLLDAQSAPLRVYVEELKPTPEGDLEILLQKWENGECAQKKIIAEKTKIPAVFKIDALNENKVLVLDTDYKKYLLFCMENSAEPEQSLACQCLVRTPEVDDEALEKFDKALKALPMHIRLSFNPTQLEEQCHIHPHPHLSF

SEQ ID NO: 21 - protein, 171 aa, synthetic construct
EAEALIVTQTMKGLDIQKVAGTWYSLAMAASDISLLDAQSAPLRVYVEELKPTPEGDLEILLQKWENGECAQKKIIAEKTKIPAVFKIDALNENKVLVLDTDYKKYLLFCMENSAEPEQSLACQCLVRTPEVDDEALEKFDKALKALPMHIRLSFNPTQLEEQCHIDDDDK

SEQ ID NO: 22 - protein, 75 aa, synthetic construct
MRFPSIFTAVLFAASSALAAPVNTTTEDETAQIPAEAVIGYSDLEGDFDVAVLPFSASIAAKEEGVSLEKREAEA

SEQ ID NO: 23 - protein, 4 aa, synthetic construct
GSGS

SEQ ID NO: 24 - protein, 10 aa, synthetic construct
GSGSHHHHHH